European Patent Specification EP 4 003 346 B1, published September 3, 2025. Title: SERPINB3 INHIBITOR FOR TUMOR TREATMENT. Applicant: UNIVERSITA' DEGLI STUDI DI PADOVA. The sequence listing filed with the application follows.

SEQUENCE LISTING (2 sequences)

SEQ ID NO: 1 - DNA, 21 bp, Artificial Sequence
  PCR sense primer
aactcctgggtggaaagtcaa

SEQ ID NO: 2 - DNA, 22 bp, Artificial Sequence
  PCR reverse primer
accaatgtggtattgctgccaa